European Patent Specification EP 3 064 512 B1, published August 30, 2023. Title: Anti-CLDN6 Antibody. Applicant: Forerunner Pharma Research Co., Ltd./The University of Tokyo. Application EP 09700588.8. The sequence listing filed with the application follows.

SEQUENCE LISTING (53 sequences)

SEQ ID NO: 1 - DNA, 27 bp, Artificial
  PCR primer
catggcctctgccggaatgcagatcct

SEQ ID NO: 2 - DNA, 27 bp, Artificial
  PCR primer
cccaaagctgttgggcactgccacttc

SEQ ID NO: 3 - DNA, 35 bp, Artificial
  PCR primer
gctaagcttaccatggcctctgccggaatgcagat

SEQ ID NO: 4 - DNA, 35 bp, Artificial
  PCR primer
gcagctagcgacgtaattcttggtagggtactcag

SEQ ID NO: 5 - DNA, 38 bp, Artificial
  PCR primer
ccggaattcccaccatggcctctgccggaatgcagatc

SEQ ID NO: 6 - DNA, 35 bp, Artificial
  PCR primer
gcggccgctcagacgtaattcttggtagggtactc

SEQ ID NO: 7 - DNA, 21 bp, Mus musculus
gggccagtggatagacagatg

SEQ ID NO: 8 - DNA, 24 bp, Mus musculus
caggggccagtggatagactgatg

SEQ ID NO: 9 - DNA, 27 bp, Mus musculus
ggcacctccagatgttaactgctcact

SEQ ID NO: 10 - DNA, 354 bp, Mus musculus
gaggtccagctgcaacagtctggacctgagttggtgaagcctggaggttcaatgaagatatcctgcaaggcttctggctactcattcactggctacaccatgaactgggtgaagcagagccatggaaagaaccttgagtggattggacttattaatccttacaatggcggtattagttacaaccagaaattcaaagacaaggccacactaactatggacaagtcatccagcacagcctacatggagctcctcagtctgacatctgaggactctgcaatctatttctgtgcaagagactataggtacgagggctttgattactggggccaagggactctggtcactgtctctgca

SEQ ID NO: 11 - protein, 118 aa, Mus musculus
EVQLQQSGPELVKPGGSMKISCKASGYSFTGYTMNWVKQSHGKNLEWIGLINPYNGGISYNQKFKDKATLTMDKSSSTAYMELLSLTSEDSAIYFCARDYRYEGFDYWGQGTLVTVSA

SEQ ID NO: 12 - DNA, 324 bp, Mus musculus
caaattgttctcacccagtctccagcaatcatgtctgcatctctaggggaacgggtcaccatgacctgtactgccagttcagttgtaatttccacttacttgcactggtaccagcagaagccaggatcctcccccaaactctggatttatagcacatccaacctggcttctggagtcccagttcgcttcagtggcagtgggtctgggacctcttactctctcacaatcagcagcatggaggctgaagatgctgccacttattactgccaccagtatcatcgttccccgtggacgttcggtggaggcaccaagctggaaatcaaa

SEQ ID NO: 13 - protein, 108 aa, Mus musculus
QIVLTQSPAIMSASLGERVTMTCTASSVVISTYLHWYQQKPGSSPKLWIYSTSNLASGVPVRFSGSGSGTSYSLTISSMEAEDAATYYCHQYHRSPWTFGGGTKLEIK

SEQ ID NO: 14 - DNA, 369 bp, Mus musculus
gaggttcagctgcagcagtctggacctgagctggtgaagcctggggcttcagtgaagatatcctgcaaggcttctggttactcatttactggctactttatgaactgggtgaaacagagccatggaaagagccttgagtggattggacgtattaatccttacaatggtgatactttctacaaccagaagttcaagggcaaggccacattaactgtagacaaatcctctaatacagcccacatggagctccggagcctgacatctgaggactctgcagtctattattgtgcaagagtcctcttccttgatttcgacgacccctatcttatggactattggggtcaaggaacctcagtcaccgtctcctca

SEQ ID NO: 15 - protein, 123 aa, Mus musculus
EVQLQQSGPELVKPGASVKISCKASGYSFTGYFMNWVKQSHGKSLEWIGRINPYNGDTFYNQKFKGKATLTVDKSSNTAHMELRSLTSEDSAVYYCARVLFLDFDDPYLMDYWGQGTSVTVSS

SEQ ID NO: 16 - DNA, 318 bp, Mus musculus
gaaaatgtgctcacccagtctccagcaatcatgtctgcaactcttggggagaaggtcaccatgagctgcagggccacctcaaatgtaaagtacatgtactggtaccagcagaagtcaggtgcctcccccaaactatggatttattacacatccaacctggcttctggagtcccagctcgcttcagtggcagtgggtctgggacctcttattctctcacaatcagcagcgtggaggctgcagatgctgccacttattactgccagcagtttactagttccccatccacgttcggtgctgggaccaagctggagctgaaa

SEQ ID NO: 17 - protein, 106 aa, Mus musculus
ENVLTQSPAIMSATLGEKVTMSCRATSNVKYMYWYQQKSGASPKLWIYYTSNLASGVPARFSGSGSGTSYSLTISSVEAADAATYYCQQFTSSPSTFGAGTKLELK

SEQ ID NO: 18 - DNA, 369 bp, Mus musculus
gaggttcagctgcagcagtctggacctgagctggtgaagcctggggcttcagtgaagatatcctgcaaggcttctggttactcatttactggctactttatgaactgggtgaagcagagccatggaaagagccttgagtggattggacgtattaatccttacaatggtgatactttctacaaccagaagttcaagggcaaggccacattaactgtagacaaatcctctagcacagcccacatggagctccggagcctgacatctgaggactctgcagtctattattgtgcaagagtcctcttccttgatttcgacgacccctatcttatggactattggggtcaaggaacctcagtcaccgtctcctca

SEQ ID NO: 19 - protein, 123 aa, Mus musculus
EVQLQQSGPELVKPGASVKISCKASGYSFTGYFMNWVKQSHGKSLEWIGRINPYNGDTFYNQKFKGKATLTVDKSSSTAHMELRSLTSEDSAVYYCARVLFLDFDDPYLMDYWGQGTSVTVSS

SEQ ID NO: 20 - DNA, 318 bp, Mus musculus; identical to SEQ ID NO: 16

SEQ ID NO: 21 - protein, 106 aa, Mus musculus; identical to SEQ ID NO: 17

SEQ ID NO: 22 - protein, 220 aa, homo sapiens
MASAGMQILGVVLTLLGWVNGLVSCALPMWKVTAFIGNSIVVAQVVWEGLWMSCVVQSTGQMQCKVYDSLLALPQDLQAARALCVIALLVALFGLLVYLAGAKCTTCVEEKDSKARLVLTSGIVFVISGVLTLIPVCWTAHAVIRDFYNPLVAEAQKRELGASLYLGWAASGLLLLGGGLLCCTCPSGGSQGPSHYMARYSTSAPAISRGPSEYPTKNYV

SEQ ID NO: 23 - DNA, 1363 bp, homo sapiens
atctccttcgcagtgcagctccttcaacctcgccatggcctctgccggaatgcagatcctgggagtcgtcctgacactgctgggctgggtgaatggcctggtctcctgtgccctgcccatgtggaaggtgaccgctttcatcggcaacagcatcgtggtggcccaggtggtgtgggagggcctgtggatgtcctgcgtggtgcagagcaccggccagatgcagtgcaaggtgtacgactcactgctggcgctgccacaggacctgcaggctgcacgtgccctctgtgtcatcgccctccttgtggccctgttcggcttgctggtctaccttgctggggccaagtgtaccacctgtgtggaggagaaggattccaaggcccgcctggtgctcacctctgggattgtctttgtcatctcaggggtcctgacgctaatccccgtgtgctggacggcgcatgccgtcatccgggacttctataaccccctggtggctgaggcccaaaagcgggagctgggggcctccctctacttgggctgggcggcctcaggccttttgttgctgggtggggggttgctgtgctgcacttgcccctcgggggggtcccagggccccagccattacatggcccgctactcaacatctgcccctgccatctctcgggggccctctgagtaccctaccaagaattacgtctgacgtggaggggaatgggggctccgctggcgctagagccatccagaagtggcagtgcccaacagctttgggatgggttcgtaccttttgtttctgcctcctgctatttttcttttgactgaggatatttaaaattcatttgaaaactgagccaaggtgttgactcagactctcacttaggctctgctgtttctcacccttggatgatggagccaaagaggggatgctttgagattctggatcttgacatgcccatcttagaagccagtcaagctatggaactaatgcggaggctgcttgctgtgctggctttgcaacaagacagactgtccccaagagttcctgctgctgctgggggctgggcttccctagatgtcactggacagctgccccccatcctactcaggtctctggagctcctctcttcacccctggaaaaacaaatgatctgttaacaaaggactgcccacctccggaacttctgacctctgtttcctccgtcctgataagacgtccaccccccagggccaggtcccagctatgtagacccccgcccccacctccaacactgcacccttctgccctgcccccctcgtctcaccccctttacactcacatttttatcaaataaagcatgttttgttagtgcaaaaaaaaaaaaaaaaaaaa

SEQ ID NO: 24 - protein, 5 aa, Mus musculus
GYTMN

SEQ ID NO: 25 - protein, 17 aa, Mus musculus
LINPYNGGISYNQKFKD

SEQ ID NO: 26 - protein, 9 aa, Mus musculus
DYRYEGFDY

SEQ ID NO: 27 - protein, 12 aa, Mus musculus
TASSVVISTYLH

SEQ ID NO: 28 - protein, 7 aa, Mus musculus
STSNLAS

SEQ ID NO: 29 - protein, 9 aa, Mus musculus
HQYHRSPWT

SEQ ID NO: 30 - protein, 5 aa, Mus musculus
GYFMN

SEQ ID NO: 31 - protein, 17 aa, Mus musculus
RINPYNGDTFYNQKFKG

SEQ ID NO: 32 - protein, 14 aa, Mus musculus
VLFLDFDDPYLMDY

SEQ ID NO: 33 - protein, 10 aa, Mus musculus
RATSNVKYMY

SEQ ID NO: 34 - protein, 7 aa, Mus musculus
YTSNLAS

SEQ ID NO: 35 - protein, 9 aa, Mus musculus
QQFTSSPST

SEQ ID NO: 36 - DNA, 357 bp, Mus musculus
gaagtgaagctggtggagtctgggggaggcttagtgaagcctggagggtccctgaaactctcctgtgcagcctctggattcactttcaatagctataccatgtcttgggttcgccagactccggcgaagaggctggagtgggtcgtaaccattagtagtggtggaggtcgcacctactatccagacagtgtgaagggccgattcaccatctccagagacaatgccaggaacaccctgtacctacaaatgagcagtctgaggtctgaagacacggccatgtattactgtataaggggggactataggtacgacgggtttgcttactggggccaggggactctggtcactgtctctaca

SEQ ID NO: 37 - protein, 119 aa, Mus musculus
EVKLVESGGGLVKPGGSLKLSCAASGFTFNSYTMSWVRQTPAKRLEWVVTISSGGGRTYYPDSVKGRFTISRDNARNTLYLQMSSLRSEDTAMYYCIRGDYRYDGFAYWGQGTLVTVST

SEQ ID NO: 38 - DNA, 321 bp, Mus musculus
gacatccagatgactcagtctccagcttccctgtctgcatctgtgggagaaactgtcaccatcacatgtcgagcaagtgagaatattgacagttatttagcatggtatcagcagaaacagggaaaatctcctcaactcctggtctatgcttcaacactcttagtagatggtgtgccatcaaggttcagtggcagtagatcaggcacacagttttctctcaaaatcaacagcctgcagtctgaagatgttgcgagatattactgtcaacattattatagtattccgtatacgttcggatcggggaccaagctggaaataaaa

SEQ ID NO: 39 - protein, 107 aa, Mus musculus
DIQMTQSPASLSASVGETVTITCRASENIDSYLAWYQQKQGKSPQLLVYASTLLVDGVPSRFSGSRSGTQFSLKINSLQSEDVARYYCQHYYSIPYTFGSGTKLEIK

SEQ ID NO: 40 - protein, 5 aa, Mus musculus
SYTMS

SEQ ID NO: 41 - protein, 17 aa, Mus musculus
TISSGGGRTYYPDSVKG

SEQ ID NO: 42 - protein, 10 aa, Mus musculus
GDYRYDGFAY

SEQ ID NO: 43 - protein, 11 aa, Mus musculus
RASENIDSYLA

SEQ ID NO: 44 - protein, 7 aa, Mus musculus
ASTLLVD

SEQ ID NO: 45 - protein, 9 aa, Mus musculus
QHYYSIPYT

SEQ ID NO: 46 - protein, 220 aa, homo sapiens
MASAGMQILGVVLTLLGWVNGLVSCALPMWKVTAFIGNSIVVAQVVWEGLWMSCVVQSTGQMQCKVYDSLLALPQDLQAARALCVIALLVALFGLLVYLAGAKCTTCVEEKDSKARLVLTSGIVFVISGVLTLIPVCWTAHAIIRDFYNPLVAEAQKRELGASLYLGWAASGLLLLGGGLLCCTCPSGGSQGPSHYMARYSTSAPAISRGPSEYPTKNYV

SEQ ID NO: 47 - DNA, 1389 bp, homo sapiens
cgacactcggcctaggaatttcccttatctccttcgcagtgcagctccttcaacctcgccatggcctctgccggaatgcagatcctgggagtcgtcctgacactgctgggctgggtgaatggcctggtctcctgtgccctgcccatgtggaaggtgaccgctttcatcggcaacagcatcgtggtggcccaggtggtgtgggagggcctgtggatgtcctgcgtggtgcagagcaccggccagatgcagtgcaaggtgtacgactcactgctggcgctgccacaggacctgcaggctgcacgtgccctctgtgtcatcgccctccttgtggccctgttcggcttgctggtctaccttgctggggccaagtgtaccacctgtgtggaggagaaggattccaaggcccgcctggtgctcacctctgggattgtctttgtcatctcaggggtcctgacgctaatccccgtgtgctggacggcgcatgccatcatccgggacttctataaccccctggtggctgaggcccaaaagcgggagctgggggcctccctctacttgggctgggcggcctcaggccttttgttgctgggtggggggttgctgtgctgcacttgcccctcgggggggtcccagggccccagccattacatggcccgctactcaacatctgcccctgccatctctcgggggccctctgagtaccctaccaagaattacgtctgacgtggaggggaatgggggctccgctggcgctagagccatccagaagtggcagtgcccaacagctttgggatgggttcgtaccttttgtttctgcctcctgctatttttcttttgactgaggatatttaaaattcatttgaaaactgagccaaggtgttgactcagactctcacttaggctctgctgtttctcacccttggatgatggagccaaagaggggatgctttgagattctggatcttgacatgcccatcttagaagccagtcaagctatggaactaatgcggaggctgcttgctgtgctggctttgcaacaagacagactgtccccaagagttcctgctgctgctgggggctgggcttccctagatgtcactggacagctgccccccatcctactcaggtctctggagctcctctcttcacccctggaaaaacaaatgatctgttaacaaaggactgcccacctccggaacttctgacctctgtttcctccgtcctgataagacgtccaccccccagggccaggtcccagctatgtagacccccgcccccacctccaacactgcacccttctgccctgcccccctcgtctcaccccctttacactcacatttttatcaaataaagcatgttttgttagtgcaaaaaaaaaaaaaaaaaaaa

SEQ ID NO: 48 - protein, 217 aa, homo sapiens
MASTGLELLGMTLAVLGWLGTLVSCALPLWKVTAFIGNSIVVAQVVWEGLWMSCVVQSTGQMQCKVYDSLLALPQDLQAARALCVIALLLALLGLLVAITGAQCTTCVEDEGAKARIVLTAGVILLLAGILVLIPVCWTAHAIIQDFYNPLVAEALKRELGASLYLGWAAAALLMLGGGLLCCTCPPPQVERPRGPRLGYSIPSRSGASGLDKRDYV

SEQ ID NO: 49 - protein, 220 aa, homo sapiens
MSMGLEITGTALAVLGWLGTIVCCALPMWRVSAFIGSNIITSQNIWEGLWMNCVVQSTGQMQCKVYDSLLALPQDLQAARALIVVAILLAAFGLLVALVGAQCTNCVQDDTAKAKITIVAGVLFLLAALLTLVPVSWSANTIIRDFYNPVVPEAQKREMGAGLYVGWAAAALQLLGGALLCCSCPPREKKYTATKVVYSAPRSTGPGASLGTGYDRKDYV

SEQ ID NO: 50 - protein, 209 aa, homo sapiens
MASMGLQVMGIALAVLGWLAVMLCCALPMWRVTAFIGSNIVTSQTIWEGLWMNCVVQSTGQMQCKVYDSLLALPQDLQAARALVIISIIVAALGVLLSVVGGKCTNCLEDESAKAKTMIVAGVVFLLAGLMVIVPVSWTAHNIIQDFYNPLVASGQKREMGASLYVGWAASGLLLLGGGLLCCNCPPRTDKPYSAKYSAARSAAASNYV

SEQ ID NO: 51 - protein, 211 aa, homo sapiens
MANAGLQLLGFILAFLGWIGAIVSTALPQWRIYSYAGDNIVTAQAMYEGLWMSCVSQSTGQIQCKVFDSLLNLSSTLQATRALMVVGILLGVIAIFVATVGMKCMKCLEDDEVQKMRMAVIGGAIFLLAGLAILVATAWYGNRIVQEFYDPMTPVNARYEFGQALFTGWAAASLCLLGGALLCCSCPRKTTSYPTPRPYPKPAPSSGKDYV

SEQ ID NO: 52 - protein, 453 aa, Artificial
  AE49-11/mIgG2a  H chain
EVQLQQSGPELVKPGASVKISCKASGYSFTGYFMNWVKQSHGKSLEWIGRINPYNGDTFYNQKFKGKATLTVDKSSSTAHMELRSLTSEDSAVYYCARVLFLDFDDPYLMDYWGQGTSVTVSSASTTAPSVYPLAPVCGDTTGSSVTLGCLVKGYFPEPVTLTWNSGSLSSGVHTFPAVLQSDLYTLSSSVTVTSSTWPSQSITCNVAHPASSTKVDKKIEPRGPTIKPCPPCKCPAPNLLGGPSVFIFPPKIKDVLMISLSPIVTCVVVDVSEDDPDVQISWFVNNVEVHTAQTQTHREDYNSTLRVVSALPIQHQDWMSGKEFKCKVNNKDLPAPIERTISKPKGSVRAPQVYVLPPPEEEMTKKQVTLTCMVTDFMPEDIYVEWTNNGKTELNYKNTEPVLDSDGSYFMYSKLRVEKKNWVERNSYSCSVVHEGLHNHHTTKSFSRTPGK

SEQ ID NO: 53 - protein, 213 aa, Artificial
  AE49-11/mIgG2a L chain
ENVLTQSPAIMSATLGEKVTMSCRATSNVKYMYWYQQKSGASPKLWIYYTSNLASGVPARFSGSGSGTSYSLTISSVEAADAATYYCQQFTSSPSTFGAGTKLELKRTVAAPTVSIFPPSSEQLTSGGASVVCFLNNFYPKDINVKWKIDGSERQNGVLNSWTDQDSKDSTYSMSSTLTLTKDEYERHNSYTCEATHKTSTSPIVKSFNRNEC